European Patent Specification EP 3 337 827 B1, published July 8, 2026. Title: TISSUE FACTOR PATHWAY INHIBITOR ANTIBODIES AND USES THEREOF. Applicant: Pfizer Inc. Pittman, Debra Apgar, James R. Juo, Zong Sean Jin, Macy Stahl, Mark Carven, Gregory J. Holsti, Matthew Benard, Susan Hett, Sunita R. Jasuja, Reema. The sequence listing filed with the application follows.

SEQUENCE LISTING (178 sequences)

SEQ ID NO: 1 - protein, 149 aa, Homo sapiens
DSEEDEEHTIITDTELPPLKLMHSFCAFKADDGPCKAIMKRFFFNIFTRQCEEFIYGGCEGNQNRFESLEECKKMCTRDNANRIIKTTLQQEKPDFCFLEEDPGICRGYITRYFYNNQTKQCERFKYGGCLGNMNNFETLEECKNICED

SEQ ID NO: 2 - protein, 254 aa, Homo sapiens
DSEEDEEHTIITDTELPPLKLMHSFCAFKADDGPCKAIMKRFFFNIFTRQCEEFIYGGCEGNQNRFESLEECKKMCTRDNANRIIKTTLQQEKPDFCFLEEDPGICRGYITRYFYNNQTKQCERFKYGGCLGNMNNFETLEECKNICEDGPNGFQVDNYGTQLNAVNNSLTPQSTKVPSLFEFHGPSWCLTPADRGLCRANENRFYYNSVIGKCRPFKYSGCGGNENNFTSKQECLRACKKGFIQRISKGGLIK

SEQ ID NO: 3 - protein, 189 aa, Homo sapiens
DAAQEPTGNNAEICLLPLDYGPCRALLLRYYYDRYTQSCRQFLYGGCEGNANNFYTWEACDDACWRIEKVPKVCRLQVSVDDQCEGSTEKYFFNLSSMTCEKFFSGGCHRNRIENRFPDEATCMGFCAPKKIPSFCYSPKDEGLCSANVTRYYFNPRYRTCDAFTYTGCGGNDNNFVSREDCKRACAKA

SEQ ID NO: 4 - protein, 146 aa, Artificial Sequence
  Synthetic Construct
LSEEADDTDSELGSMKPLHTFCAMKADDGPCKAMIRSYFFNMYTHQCEEFIYGGCEGNENRFDTLEECKKTCIPGYEKTAVKAASGAERPDFCFLEEDPGLCRGYMKRYLYNNQTKQCERFVYGGCLGNRNNFETLDECKKICENP

SEQ ID NO: 5 - protein, 149 aa, Artificial Sequence
  Synthetic Construct
DSEEDEEYTIITDTELPPLKLMHSFCAFKPDDGPCKAIMKRFFFNIFTRQCEEFIYGGCGGNQNRFESMEECKKVCTRDNVNRIIQTALQKEKPDFCFLEEDPGICRGYITRYFYNNQSKQCERFKYGGCLGNMNNFETLEECKNTCED

SEQ ID NO: 6 - protein, 149 aa, Artificial Sequence
  Synthetic Construct
AAEEDEEFTNITDIKPPLQKPTHSFCAMKVDDGPCRAYIKRFFFNILTHQCEEFIYGGCEGNENRFESLEECKEKCARDYPKMTTKLTFQKGKPDFCFLEEDPGICRGYITRYFYNNQSKQCERFKYGGCLGNLNNFESLEECKNTCEN

SEQ ID NO: 7 - protein, 148 aa, Artificial Sequence
  Synthetic Construct
LPEEDDDTINTDSELRPMKPLHTFCAMKAEDGPCKAMIRSYYFNMNSHQCEEFIYGGCRGNKNRFDTLEECRKTCIPGYKKTTIKTTSGAEKPDFCFLEEDPGICRGFMTRYFYNNQSKQCEQFKYGGCLGNSNNFETLEECRNTCED

SEQ ID NO: 8 - protein, 35 aa, Artificial Sequence
  Synthetic Construct
GGGSGGGLNDIFEAQKIEWHEGGPPHHHHHHHHHH

SEQ ID NO: 9 - protein, 20 aa, Artificial Sequence
  Synthetic Construct
METDTLLLWVLLLWVPGSTG

SEQ ID NO: 10 - protein, 11 aa, Artificial Sequence
  Synthetic Construct
RASQGISSSLA

SEQ ID NO: 11 - protein, 7 aa, Artificial Sequence
  Synthetic Construct
AASTLQS

SEQ ID NO: 12 - protein, 9 aa, Artificial Sequence
  Synthetic Construct
QQLDSYPLS

SEQ ID NO: 13 - protein, 107 aa, Artificial Sequence
  Synthetic Construct
AIQLTQSPSSLSASVGDRVTITCRASQGISSSLAWYQQKPGKAPKLLIYAASTLQSGVPSRFSGSGSGTDFTLTISSLQPEDFATYYCQQLDSYPLSFGQGTKLEIK

SEQ ID NO: 14 - protein, 107 aa, Homo sapiens [sequence omitted]

SEQ ID NO: 15 - protein, 214 aa, Artificial Sequence
  Synthetic Construct
AIQLTQSPSSLSASVGDRVTITCRASQGISSSLAWYQQKPGKAPKLLIYAASTLQSGVPSRFSGSGSGTDFTLTISSLQPEDFATYYCQQLDSYPLSFGQGTKLEIKRTVAAPSVFIFPPSDEQLKSGTASVVCLLNNFYPREAKVQWKVDNALQSGNSQESVTEQDSKDSTYSLSSTLTLSKADYEKHKVYACEVTHQGLSSPVTKSFNRGEC

SEQ ID NO: 16 - protein, 10 aa, Artificial Sequence
  Synthetic Construct
GYTFTGYYMH

SEQ ID NO: 17 - protein, 17 aa, Artificial Sequence
  Synthetic Construct
WINPNSGGTNYAQKFQG

SEQ ID NO: 18 - protein, 16 aa, Artificial Sequence
  Synthetic Construct
GIARLQWLPTEADFDY

SEQ ID NO: 19 - protein, 125 aa, Artificial Sequence
  Synthetic Construct
QVQLVQSGAEVKKPGASVKVSCKASGYTFTGYYMHWVRQAPGQGLEWMGWINPNSGGTNYAQKFQGRVTMTRDTSISTAYMELSRLRSDDTAVYYCARGIARLQWLPTEADFDYWGQGTLVTVSS

SEQ ID NO: 20 - protein, 329 aa, Homo sapiens
ASTKGPSVFPLAPSSKSTSGGTAALGCLVKDYFPEPVTVSWNSGALTSGVHTFPAVLQSSGLYSLSSVVTVPSSSLGTQTYICNVNHKPSNTKVDKKVEPKSCDKTHTCPPCPAPEAAGAPSVFLFPPKPKDTLMISRTPEVTCVVVDVSHEDPEVKFNWYVDGVEVHNAKTKPREEQYNSTYRVVSVLTVLHQDWLNGKEYKCKVSNKALPAPIEKTISKAKGQPREPQVYTLPPSREEMTKNQVSLTCLVKGFYPSDIAVEWESNGQPENNYKTTPPVLDSDGSFFLYSKLTVDKSRWQQGNVFSCSVMHEALHNHYTQKSLSLSPG

SEQ ID NO: 21 - protein, 454 aa, Artificial Sequence
  Synthetic Construct
QVQLVQSGAEVKKPGASVKVSCKASGYTFTGYYMHWVRQAPGQGLEWMGWINPNSGGTNYAQKFQGRVTMTRDTSISTAYMELSRLRSDDTAVYYCARGIARLQWLPTEADFDYWGQGTLVTVSSASTKGPSVFPLAPSSKSTSGGTAALGCLVKDYFPEPVTVSWNSGALTSGVHTFPAVLQSSGLYSLSSVVTVPSSSLGTQTYICNVNHKPSNTKVDKKVEPKSCDKTHTCPPCPAPEAAGAPSVFLFPPKPKDTLMISRTPEVTCVVVDVSHEDPEVKFNWYVDGVEVHNAKTKPREEQYNSTYRVVSVLTVLHQDWLNGKEYKCKVSNKALPAPIEKTISKAKGQPREPQVYTLPPSREEMTKNQVSLTCLVKGFYPSDIAVEWESNGQPENNYKTTPPVLDSDGSFFLYSKLTVDKSRWQQGNVFSCSVMHEALHNHYTQKSLSLSPG

SEQ ID NO: 22 - protein, 14 aa, Artificial Sequence
  Synthetic Construct
TGSSSNIGAGYDVH

SEQ ID NO: 23 - protein, 7 aa, Artificial Sequence
  Synthetic Construct
GNSNRPS

SEQ ID NO: 24 - protein, 12 aa, Artificial Sequence
  Synthetic Construct
QSYDSSLSGSVV

SEQ ID NO: 25 - protein, 113 aa, Artificial Sequence
  Synthetic Construct
QSVLTQPPSVSGAPGQRVTISCTGSSSNIGAGYDVHWYQQLPGTAPKLLIYGNSNRPSGVPDRFSGSKSGTSASLAITGLQAEDEADFYCQSYDSSLSGSVVFGGGTKVTVLG

SEQ ID NO: 26 - protein, 105 aa, Homo sapiens
QPKAAPSVTLFPPSSEELQANKATLVCLISDFYPGAVTVAWKADSSPVKAGVETTTPSKQSNNKYAASSYLSLTPEQWKSHRSYSCQVTHEGSTVEKTVAPTECS

SEQ ID NO: 27 - protein, 218 aa, Artificial Sequence
  Synthetic Construct
QSVLTQPPSVSGAPGQRVTISCTGSSSNIGAGYDVHWYQQLPGTAPKLLIYGNSNRPSGVPDRFSGSKSGTSASLAITGLQAEDEADFYCQSYDSSLSGSVVFGGGTKVTVLGQPKAAPSVTLFPPSSEELQANKATLVCLISDFYPGAVTVAWKADSSPVKAGVETTTPSKQSNNKYAASSYLSLTPEQWKSHRSYSCQVTHEGSTVEKTVAPTECS

SEQ ID NO: 28 - protein, 10 aa, Artificial Sequence
  Synthetic Construct
GFTFSSYAMS

SEQ ID NO: 29 - protein, 17 aa, Artificial Sequence
  Synthetic Construct
AISGSGGSTYYADSVKG

SEQ ID NO: 30 - protein, 11 aa, Artificial Sequence
  Synthetic Construct
LGATSLSAFDI

SEQ ID NO: 31 - protein, 120 aa, Artificial Sequence
  Synthetic Construct
QVQLVESGGGLVQPGGSLRLSCAASGFTFSSYAMSWVRQAPGKGLEWVSAISGSGGSTYYADSVKGRFTISRDNSKNTLYLQMNSLRAEDTAVYYCAILGATSLSAFDIWGQGTMVTVSS

SEQ ID NO: 32 - protein, 449 aa, Artificial Sequence
  Synthetic Construct
QVQLVESGGGLVQPGGSLRLSCAASGFTFSSYAMSWVRQAPGKGLEWVSAISGSGGSTYYADSVKGRFTISRDNSKNTLYLQMNSLRAEDTAVYYCAILGATSLSAFDIWGQGTMVTVSSASTKGPSVFPLAPSSKSTSGGTAALGCLVKDYFPEPVTVSWNSGALTSGVHTFPAVLQSSGLYSLSSVVTVPSSSLGTQTYICNVNHKPSNTKVDKKVEPKSCDKTHTCPPCPAPEAAGAPSVFLFPPKPKDTLMISRTPEVTCVVVDVSHEDPEVKFNWYVDGVEVHNAKTKPREEQYNSTYRVVSVLTVLHQDWLNGKEYKCKVSNKALPAPIEKTISKAKGQPREPQVYTLPPSREEMTKNQVSLTCLVKGFYPSDIAVEWESNGQPENNYKTTPPVLDSDGSFFLYSKLTVDKSRWQQGNVFSCSVMHEALHNHYTQKSLSLSPG

SEQ ID NO: 33 - protein, 14 aa, Artificial Sequence
  Synthetic Construct
TGSSSNIGAGYDVH

SEQ ID NO: 34 - protein, 7 aa, Artificial Sequence
  Synthetic Construct
GNSNRPS

SEQ ID NO: 35 - protein, 12 aa, Artificial Sequence
  Synthetic Construct
QSYDSSLSGSGV

SEQ ID NO: 36 - protein, 113 aa, Artificial Sequence
  Synthetic Construct
QSVLTQPPSVSGAPGQRVTISCTGSSSNIGAGYDVHWYQQLPGTAPKLLIYGNSNRPSGVPDRFSGSKSGTSASLAITGLQAEDEADYYCQSYDSSLSGSGVFGGGTKLTVLG

SEQ ID NO: 37 - protein, 218 aa, Artificial Sequence
  Synthetic Construct
QSVLTQPPSVSGAPGQRVTISCTGSSSNIGAGYDVHWYQQLPGTAPKLLIYGNSNRPSGVPDRFSGSKSGTSASLAITGLQAEDEADYYCQSYDSSLSGSGVFGGGTKLTVLGQPKAAPSVTLFPPSSEELQANKATLVCLISDFYPGAVTVAWKADSSPVKAGVETTTPSKQSNNKYAASSYLSLTPEQWKSHRSYSCQVTHEGSTVEKTVAPTECS

SEQ ID NO: 38 - protein, 10 aa, Artificial Sequence
  Synthetic Construct
GFTFSSYAMS

SEQ ID NO: 39 - protein, 17 aa, Artificial Sequence
  Synthetic Construct
AISGSGGSTYYADSVKG

SEQ ID NO: 40 - protein, 11 aa, Artificial Sequence
  Synthetic Construct
LGATSLSAFDI

SEQ ID NO: 41 - protein, 120 aa, Artificial Sequence; identical to SEQ ID NO: 31
  Synthetic Construct

SEQ ID NO: 42 - protein, 449 aa, Artificial Sequence; identical to SEQ ID NO: 32
  Synthetic Construct

SEQ ID NO: 43 - protein, 13 aa, Artificial Sequence
  Synthetic Construct
SGSTSNIGTMYVH

SEQ ID NO: 44 - protein, 7 aa, Artificial Sequence
  Synthetic Construct
RNNHRPS

SEQ ID NO: 45 - protein, 11 aa, Artificial Sequence
  Synthetic Construct
LAWDDTLRAYV

SEQ ID NO: 46 - protein, 111 aa, Artificial Sequence
  Synthetic Construct
QSVLTQPPSVSGTPGQRVTISCSGSTSNIGTMYVHWYQHVPGTAPKLLIYRNNHRPSGVPDRFSGSKSGTSGSLAISGLRSEDEADYYCLAWDDTLRAYVFGTGTKVTVLG

SEQ ID NO: 47 - protein, 216 aa, Artificial Sequence
  Synthetic Construct
QSVLTQPPSVSGTPGQRVTISCSGSTSNIGTMYVHWYQHVPGTAPKLLIYRNNHRPSGVPDRFSGSKSGTSGSLAISGLRSEDEADYYCLAWDDTLRAYVFGTGTKVTVLGQPKAAPSVTLFPPSSEELQANKATLVCLISDFYPGAVTVAWKADSSPVKAGVETTTPSKQSNNKYAASSYLSLTPEQWKSHRSYSCQVTHEGSTVEKTVAPTECS

SEQ ID NO: 48 - protein, 10 aa, Artificial Sequence
  Synthetic Construct
GLTIDNYAMQ

SEQ ID NO: 49 - protein, 17 aa, Artificial Sequence
  Synthetic Construct
GISGNSRSIGYADSVKG

SEQ ID NO: 50 - protein, 7 aa, Artificial Sequence
  Synthetic Construct
FLHESDY

SEQ ID NO: 51 - protein, 116 aa, Artificial Sequence
  Synthetic Construct
EVQLVESGGGSVQPGRSLRLSCAVSGLTIDNYAMQWVRQRPGKGLEWVSGISGNSRSIGYADSVKGRLTISRDNAKNSLYLQIDSLRADDTALYYCAIFLHESDYWGQGTLVTVSS

SEQ ID NO: 52 - protein, 445 aa, Artificial Sequence
  Synthetic Construct
EVQLVESGGGSVQPGRSLRLSCAVSGLTIDNYAMQWVRQRPGKGLEWVSGISGNSRSIGYADSVKGRLTISRDNAKNSLYLQIDSLRADDTALYYCAIFLHESDYWGQGTLVTVSSASTKGPSVFPLAPSSKSTSGGTAALGCLVKDYFPEPVTVSWNSGALTSGVHTFPAVLQSSGLYSLSSVVTVPSSSLGTQTYICNVNHKPSNTKVDKKVEPKSCDKTHTCPPCPAPEAAGAPSVFLFPPKPKDTLMISRTPEVTCVVVDVSHEDPEVKFNWYVDGVEVHNAKTKPREEQYNSTYRVVSVLTVLHQDWLNGKEYKCKVSNKALPAPIEKTISKAKGQPREPQVYTLPPSREEMTKNQVSLTCLVKGFYPSDIAVEWESNGQPENNYKTTPPVLDSDGSFFLYSKLTVDKSRWQQGNVFSCSVMHEALHNHYTQKSLSLSPG

SEQ ID NO: 53 - protein, 14 aa, Artificial Sequence
  Synthetic Construct
TGSSSNLGADYDVQ

SEQ ID NO: 54 - protein, 7 aa, Artificial Sequence
  Synthetic Construct
GNNNRPS

SEQ ID NO: 55 - protein, 12 aa, Artificial Sequence
  Synthetic Construct
QSYDRSLSGSMV

SEQ ID NO: 56 - protein, 113 aa, Artificial Sequence
  Synthetic Construct
QSVLTQPPSLSGAPGQRVTISCTGSSSNLGADYDVQWYQQLPGTAPKLLIFGNNNRPSGVPDRFSGSRSGTSASLAITGLQAEDEANYYCQSYDRSLSGSMVFGGGTKLTVLG

SEQ ID NO: 57 - protein, 218 aa, Artificial Sequence
  Synthetic Construct
QSVLTQPPSLSGAPGQRVTISCTGSSSNLGADYDVQWYQQLPGTAPKLLIFGNNNRPSGVPDRFSGSRSGTSASLAITGLQAEDEANYYCQSYDRSLSGSMVFGGGTKLTVLGQPKAAPSVTLFPPSSEELQANKATLVCLISDFYPGAVTVAWKADSSPVKAGVETTTPSKQSNNKYAASSYLSLTPEQWKSHRSYSCQVTHEGSTVEKTVAPTECS

SEQ ID NO: 58 - protein, 10 aa, Artificial Sequence
  Synthetic Construct
GFTFSSYAMS

SEQ ID NO: 59 - protein, 17 aa, Artificial Sequence
  Synthetic Construct
AISGSGGSTYYADSVKG

SEQ ID NO: 60 - protein, 9 aa, Artificial Sequence
  Synthetic Construct
NGAAAAWDY

SEQ ID NO: 61 - protein, 118 aa, Artificial Sequence
  Synthetic Construct
EVQLVESGGGLVQPGGSLRLSCAASGFTFSSYAMSWVRQAPGKGLEWVSAISGSGGSTYYADSVKGRFTISRDNSKNTLYLQMNSLRAEDTAVYYCANNGAAAAWDYWGQGTLVTVSS

SEQ ID NO: 62 - protein, 447 aa, Artificial Sequence
  Synthetic Construct
EVQLVESGGGLVQPGGSLRLSCAASGFTFSSYAMSWVRQAPGKGLEWVSAISGSGGSTYYADSVKGRFTISRDNSKNTLYLQMNSLRAEDTAVYYCANNGAAAAWDYWGQGTLVTVSSASTKGPSVFPLAPSSKSTSGGTAALGCLVKDYFPEPVTVSWNSGALTSGVHTFPAVLQSSGLYSLSSVVTVPSSSLGTQTYICNVNHKPSNTKVDKKVEPKSCDKTHTCPPCPAPEAAGAPSVFLFPPKPKDTLMISRTPEVTCVVVDVSHEDPEVKFNWYVDGVEVHNAKTKPREEQYNSTYRVVSVLTVLHQDWLNGKEYKCKVSNKALPAPIEKTISKAKGQPREPQVYTLPPSREEMTKNQVSLTCLVKGFYPSDIAVEWESNGQPENNYKTTPPVLDSDGSFFLYSKLTVDKSRWQQGNVFSCSVMHEALHNHYTQKSLSLSPG

SEQ ID NO: 63 - protein, 120 aa, Artificial Sequence
  Synthetic Construct
EVQLLESGGGLVQPGGSLRLSCAASGFTFSSYAMSWVRQAPGKGLEWVSAISGSGGSTYYADSVKGRFTISRDNSKNTLYLQMNSLRAEDTAVYYCAILGATSLSAFDIWGQGTMVTVSS

SEQ ID NO: 64 - protein, 449 aa, Artificial Sequence
  Synthetic Construct
EVQLLESGGGLVQPGGSLRLSCAASGFTFSSYAMSWVRQAPGKGLEWVSAISGSGGSTYYADSVKGRFTISRDNSKNTLYLQMNSLRAEDTAVYYCAILGATSLSAFDIWGQGTMVTVSSASTKGPSVFPLAPSSKSTSGGTAALGCLVKDYFPEPVTVSWNSGALTSGVHTFPAVLQSSGLYSLSSVVTVPSSSLGTQTYICNVNHKPSNTKVDKKVEPKSCDKTHTCPPCPAPEAAGAPSVFLFPPKPKDTLMISRTPEVTCVVVDVSHEDPEVKFNWYVDGVEVHNAKTKPREEQYNSTYRVVSVLTVLHQDWLNGKEYKCKVSNKALPAPIEKTISKAKGQPREPQVYTLPPSREEMTKNQVSLTCLVKGFYPSDIAVEWESNGQPENNYKTTPPVLDSDGSFFLYSKLTVDKSRWQQGNVFSCSVMHEALHNHYTQKSLSLSPG

SEQ ID NO: 65 - protein, 120 aa, Artificial Sequence
  Synthetic Construct
EVQLLESGGGLVQPGGSLRLSCAASGFTFSSYAMSWVRQAPGKGLEWVSAISGSGGSTYYADSVKGRFTISRDNSKNTLYLQMNSLRAEDTAVYYCAKLGATSLSAFDIWGQGTMVTVSS

SEQ ID NO: 66 - protein, 449 aa, Artificial Sequence
  Synthetic Construct
EVQLLESGGGLVQPGGSLRLSCAASGFTFSSYAMSWVRQAPGKGLEWVSAISGSGGSTYYADSVKGRFTISRDNSKNTLYLQMNSLRAEDTAVYYCAKLGATSLSAFDIWGQGTMVTVSSASTKGPSVFPLAPSSKSTSGGTAALGCLVKDYFPEPVTVSWNSGALTSGVHTFPAVLQSSGLYSLSSVVTVPSSSLGTQTYICNVNHKPSNTKVDKKVEPKSCDKTHTCPPCPAPEAAGAPSVFLFPPKPKDTLMISRTPEVTCVVVDVSHEDPEVKFNWYVDGVEVHNAKTKPREEQYNSTYRVVSVLTVLHQDWLNGKEYKCKVSNKALPAPIEKTISKAKGQPREPQVYTLPPSREEMTKNQVSLTCLVKGFYPSDIAVEWESNGQPENNYKTTPPVLDSDGSFFLYSKLTVDKSRWQQGNVFSCSVMHEALHNHYTQKSLSLSPG

SEQ ID NO: 67 - protein, 116 aa, Artificial Sequence
  Synthetic Construct
EVQLVESGGGLVQPGRSLRLSCAVSGLTIDNYAMQWVRQAPGKGLEWVSGISGNSRSIGYADSVKGRFTISRDNAKNSLYLQMNSLRAEDTALYYCAIFLHESDYWGQGTLVTVSS

SEQ ID NO: 68 - protein, 445 aa, Artificial Sequence
  Synthetic Construct
EVQLVESGGGLVQPGRSLRLSCAVSGLTIDNYAMQWVRQAPGKGLEWVSGISGNSRSIGYADSVKGRFTISRDNAKNSLYLQMNSLRAEDTALYYCAIFLHESDYWGQGTLVTVSSASTKGPSVFPLAPSSKSTSGGTAALGCLVKDYFPEPVTVSWNSGALTSGVHTFPAVLQSSGLYSLSSVVTVPSSSLGTQTYICNVNHKPSNTKVDKKVEPKSCDKTHTCPPCPAPEAAGAPSVFLFPPKPKDTLMISRTPEVTCVVVDVSHEDPEVKFNWYVDGVEVHNAKTKPREEQYNSTYRVVSVLTVLHQDWLNGKEYKCKVSNKALPAPIEKTISKAKGQPREPQVYTLPPSREEMTKNQVSLTCLVKGFYPSDIAVEWESNGQPENNYKTTPPVLDSDGSFFLYSKLTVDKSRWQQGNVFSCSVMHEALHNHYTQKSLSLSPG

SEQ ID NO: 69 - protein, 116 aa, Artificial Sequence
  Synthetic Construct
EVQLVESGGGLVQPGRSLRLSCAASGLTIDNYAMQWVRQAPGKGLEWVSGISGNSRSIGYADSVKGRLTISRDNAKNSLYLQMNSLRAEDTALYYCAIFLHESDYWGQGTLVTVSS

SEQ ID NO: 70 - protein, 445 aa, Artificial Sequence
  Synthetic Construct
EVQLVESGGGLVQPGRSLRLSCAASGLTIDNYAMQWVRQAPGKGLEWVSGISGNSRSIGYADSVKGRLTISRDNAKNSLYLQMNSLRAEDTALYYCAIFLHESDYWGQGTLVTVSSASTKGPSVFPLAPSSKSTSGGTAALGCLVKDYFPEPVTVSWNSGALTSGVHTFPAVLQSSGLYSLSSVVTVPSSSLGTQTYICNVNHKPSNTKVDKKVEPKSCDKTHTCPPCPAPEAAGAPSVFLFPPKPKDTLMISRTPEVTCVVVDVSHEDPEVKFNWYVDGVEVHNAKTKPREEQYNSTYRVVSVLTVLHQDWLNGKEYKCKVSNKALPAPIEKTISKAKGQPREPQVYTLPPSREEMTKNQVSLTCLVKGFYPSDIAVEWESNGQPENNYKTTPPVLDSDGSFFLYSKLTVDKSRWQQGNVFSCSVMHEALHNHYTQKSLSLSPG

SEQ ID NO: 71 - protein, 111 aa, Artificial Sequence
  Synthetic Construct
QSVLTQPPSASGTPGQRVTISCSGSTSNIGTMYVHWYQHLPGTAPKLLIYRNNHRPSGVPDRFSGSKSGTSASLAISGLRSEDEADYYCLAWDDTLRAYVFGTGTKVTVLG

SEQ ID NO: 72 - protein, 216 aa, Artificial Sequence
  Synthetic Construct
QSVLTQPPSASGTPGQRVTISCSGSTSNIGTMYVHWYQHLPGTAPKLLIYRNNHRPSGVPDRFSGSKSGTSASLAISGLRSEDEADYYCLAWDDTLRAYVFGTGTKVTVLGQPKAAPSVTLFPPSSEELQANKATLVCLISDFYPGAVTVAWKADSSPVKAGVETTTPSKQSNNKYAASSYLSLTPEQWKSHRSYSCQVTHEGSTVEKTVAPTECS

SEQ ID NO: 73 - protein, 111 aa, Artificial Sequence
  Synthetic Construct
QSVLTQPPSASGTPGQRVTISCSGSTSNIGTMYVHWYQQLPGTAPKLLIYRNNHRPSGVPDRFSGSKSGTSGSLAISGLRSEDEADYYCLAWDDTLRAYVFGTGTKVTVLG

SEQ ID NO: 74 - protein, 216 aa, Artificial Sequence
  Synthetic Construct
QSVLTQPPSASGTPGQRVTISCSGSTSNIGTMYVHWYQQLPGTAPKLLIYRNNHRPSGVPDRFSGSKSGTSGSLAISGLRSEDEADYYCLAWDDTLRAYVFGTGTKVTVLGQPKAAPSVTLFPPSSEELQANKATLVCLISDFYPGAVTVAWKADSSPVKAGVETTTPSKQSNNKYAASSYLSLTPEQWKSHRSYSCQVTHEGSTVEKTVAPTECS

SEQ ID NO: 75 - protein, 111 aa, Artificial Sequence
  Synthetic Construct
QSVLTQPPSASGTPGQRVTISCSGSTSNIGTMYVHWYQHLPGTAPKLLIYRNNHRPSGVPDRFSGSKSGTSGSLAISGLRSEDEADYYCLAWDDTLRAYVFGTGTKVTVLG

SEQ ID NO: 76 - protein, 216 aa, Artificial Sequence
  Synthetic Construct
QSVLTQPPSASGTPGQRVTISCSGSTSNIGTMYVHWYQHLPGTAPKLLIYRNNHRPSGVPDRFSGSKSGTSGSLAISGLRSEDEADYYCLAWDDTLRAYVFGTGTKVTVLGQPKAAPSVTLFPPSSEELQANKATLVCLISDFYPGAVTVAWKADSSPVKAGVETTTPSKQSNNKYAASSYLSLTPEQWKSHRSYSCQVTHEGSTVEKTVAPTECS

SEQ ID NO: 77 - protein, 111 aa, Artificial Sequence
  Synthetic Construct
QSVLTQPPSASGTPGQRVTISCSGSTSNIGTMYVHWYQQLPGTAPKLLIYRNNHRPSGVPDRFSGSKSGTSASLAISGLRSEDEADYYCLAWDDTLRAYVFGTGTKVTVLG

SEQ ID NO: 78 - protein, 216 aa, Artificial Sequence
  Synthetic Construct
QSVLTQPPSASGTPGQRVTISCSGSTSNIGTMYVHWYQQLPGTAPKLLIYRNNHRPSGVPDRFSGSKSGTSASLAISGLRSEDEADYYCLAWDDTLRAYVFGTGTKVTVLGQPKAAPSVTLFPPSSEELQANKATLVCLISDFYPGAVTVAWKADSSPVKAGVETTTPSKQSNNKYAASSYLSLTPEQWKSHRSYSCQVTHEGSTVEKTVAPTECS

SEQ ID NO: 79 - protein, 116 aa, Artificial Sequence
  Synthetic Construct
EVQLVESGGGLVQPGRSLRLSCAVSGLTIDNYAMQWVRQAPGKGLEWVSGISGNSRSIGYADSVKGRLTISRDNAKNSLYLQMNSLRAEDTALYYCAIFLHESDYWGQGTLVTVSS

SEQ ID NO: 80 - protein, 445 aa, Artificial Sequence
  Synthetic Construct
EVQLVESGGGLVQPGRSLRLSCAVSGLTIDNYAMQWVRQAPGKGLEWVSGISGNSRSIGYADSVKGRLTISRDNAKNSLYLQMNSLRAEDTALYYCAIFLHESDYWGQGTLVTVSSASTKGPSVFPLAPSSKSTSGGTAALGCLVKDYFPEPVTVSWNSGALTSGVHTFPAVLQSSGLYSLSSVVTVPSSSLGTQTYICNVNHKPSNTKVDKKVEPKSCDKTHTCPPCPAPEAAGAPSVFLFPPKPKDTLMISRTPEVTCVVVDVSHEDPEVKFNWYVDGVEVHNAKTKPREEQYNSTYRVVSVLTVLHQDWLNGKEYKCKVSNKALPAPIEKTISKAKGQPREPQVYTLPPSREEMTKNQVSLTCLVKGFYPSDIAVEWESNGQPENNYKTTPPVLDSDGSFFLYSKLTVDKSRWQQGNVFSCSVMHEALHNHYTQKSLSLSPG

SEQ ID NO: 81 - protein, 11 aa, Artificial Sequence
  Synthetic Construct
KASQDVHTAVA

SEQ ID NO: 82 - protein, 7 aa, Artificial Sequence
  Synthetic Construct
WASTRHT

SEQ ID NO: 83 - protein, 9 aa, Artificial Sequence
  Synthetic Construct
QQHYTTPYT

SEQ ID NO: 84 - protein, 107 aa, Artificial Sequence
  Synthetic Construct
DIVMTQSHKFMSTSVGDRVSITCKASQDVHTAVAWYQQKPGQSPRLLIYWASTRHTGVPDRFTGCGSGTDYTLTISSVQAEDLALYYCQQHYTTPYTFGGGTKLEMK

SEQ ID NO: 85 - protein, 106 aa, Artificial Sequence
  Synthetic Construct
ADAAPTVSIFPPSSEQLTSGGASVVCFLNNFYPKDINVKWKIDGSERQNGVLNSWTDQDSKDSTYSMSSTLTLTKDEYERHNSYTCEATHKTSTSPIVKSFNRNEC

SEQ ID NO: 86 - protein, 213 aa, Artificial Sequence
  Synthetic Construct
DIVMTQSHKFMSTSVGDRVSITCKASQDVHTAVAWYQQKPGQSPRLLIYWASTRHTGVPDRFTGCGSGTDYTLTISSVQAEDLALYYCQQHYTTPYTFGGGTKLEMKADAAPTVSIFPPSSEQLTSGGASVVCFLNNFYPKDINVKWKIDGSERQNGVLNSWTDQDSKDSTYSMSSTLTLTKDEYERHNSYTCEATHKTSTSPIVKSFNRNEC

SEQ ID NO: 87 - protein, 10 aa, Artificial Sequence
  Synthetic Construct
GYTFTDYNLD

SEQ ID NO: 88 - protein, 17 aa, Artificial Sequence
  Synthetic Construct
DINPINGATLYNQKFKG

SEQ ID NO: 89 - protein, 10 aa, Artificial Sequence
  Synthetic Construct
YYGDYDAMDY

SEQ ID NO: 90 - protein, 119 aa, Artificial Sequence
  Synthetic Construct
EVLLQQSGPELVKPGASVKIPCKASGYTFTDYNLDWVKQSHGKSLEWIGDINPINGATLYNQKFKGKATLTVDQSSSTAYMELRSLTSEDTAVYYCSIYYGDYDAMDYWGQGASVTVSS

SEQ ID NO: 91 - protein, 324 aa, Artificial Sequence
  Synthetic Construct
AKTTPPSVYPLAPGSAAQTNSMVTLGCLVKGYFPEPVTVTWNSGSLSSGVHTFPAVLQSDLYTLSSSVTVPSSTWPSETVTCNVAHPASSTKVDKKIVPRDCGCKPCICTVPEVSSVFIFPPKPKDVLTITLTPKVTCVVVDISKDDPEVQFSWFVDDVEVHTAQTQPREEQFNSTFRSVSELPIMHQDWLNGKEFKCRVNSAAFPAPIEKTISKTKGRPKAPQVYTIPPPKEQMAKDKVSLTCMITDFFPEDITVEWQWNGQPAENYKNTQPIMDTDGSYFVYSKLNVQKSNWEAGNTFTCSVLHEGLHNHHTEKSLSHSPGK

SEQ ID NO: 92 - protein, 443 aa, Artificial Sequence
  Synthetic Construct
EVLLQQSGPELVKPGASVKIPCKASGYTFTDYNLDWVKQSHGKSLEWIGDINPINGATLYNQKFKGKATLTVDQSSSTAYMELRSLTSEDTAVYYCSIYYGDYDAMDYWGQGASVTVSSAKTTPPSVYPLAPGSAAQTNSMVTLGCLVKGYFPEPVTVTWNSGSLSSGVHTFPAVLQSDLYTLSSSVTVPSSTWPSETVTCNVAHPASSTKVDKKIVPRDCGCKPCICTVPEVSSVFIFPPKPKDVLTITLTPKVTCVVVDISKDDPEVQFSWFVDDVEVHTAQTQPREEQFNSTFRSVSELPIMHQDWLNGKEFKCRVNSAAFPAPIEKTISKTKGRPKAPQVYTIPPPKEQMAKDKVSLTCMITDFFPEDITVEWQWNGQPAENYKNTQPIMDTDGSYFVYSKLNVQKSNWEAGNTFTCSVLHEGLHNHHTEKSLSHSPGK

SEQ ID NO: 93 - protein, 214 aa, Artificial Sequence
  Synthetic Construct
DIVMTQSHKFMSTSVGDRVSITCKASQDVHTAVAWYQQKPGQSPRLLIYWASTRHTGVPDRFTGCGSGTDYTLTISSVQAEDLALYYCQQHYTTPYTFGGGTKLEMKRTVAAPSVFIFPPSDEQLKSGTASVVCLLNNFYPREAKVQWKVDNALQSGNSQESVTEQDSKDSTYSLSSTLTLSKADYEKHKVYACEVTHQGLSSPVTKSFNRGEC

SEQ ID NO: 94 - protein, 448 aa, Artificial Sequence
  Synthetic Construct
EVLLQQSGPELVKPGASVKIPCKASGYTFTDYNLDWVKQSHGKSLEWIGDINPINGATLYNQKFKGKATLTVDQSSSTAYMELRSLTSEDTAVYYCSIYYGDYDAMDYWGQGASVTVSSASTKGPSVFPLAPSSKSTSGGTAALGCLVKDYFPEPVTVSWNSGALTSGVHTFPAVLQSSGLYSLSSVVTVPSSSLGTQTYICNVNHKPSNTKVDKKVEPKSCDKTHTCPPCPAPEAAGAPSVFLFPPKPKDTLMISRTPEVTCVVVDVSHEDPEVKFNWYVDGVEVHNAKTKPREEQYNSTYRVVSVLTVLHQDWLNGKEYKCKVSNKALPAPIEKTISKAKGQPREPQVYTLPPSREEMTKNQVSLTCLVKGFYPSDIAVEWESNGQPENNYKTTPPVLDSDGSFFLYSKLTVDKSRWQQGNVFSCSVMHEALHNHYTQKSLSLSPG

SEQ ID NO: 95 - protein, 119 aa, Artificial Sequence
  Synthetic Construct
EVQLVESGGGLVQPGGSLRLSCAASGYTFTDYNLDWVRQAPGKGLEWVADINPINGATLYNQKFKGRFTISRDNAKNSLYLQMNSLRAEDTAVYYCARYYGDYDAMDYWGQGTLVTVSS

SEQ ID NO: 96 - protein, 448 aa, Artificial Sequence
  Synthetic Construct
EVQLVESGGGLVQPGGSLRLSCAASGYTFTDYNLDWVRQAPGKGLEWVADINPINGATLYNQKFKGRFTISRDNAKNSLYLQMNSLRAEDTAVYYCARYYGDYDAMDYWGQGTLVTVSSASTKGPSVFPLAPSSKSTSGGTAALGCLVKDYFPEPVTVSWNSGALTSGVHTFPAVLQSSGLYSLSSVVTVPSSSLGTQTYICNVNHKPSNTKVDKKVEPKSCDKTHTCPPCPAPEAAGAPSVFLFPPKPKDTLMISRTPEVTCVVVDVSHEDPEVKFNWYVDGVEVHNAKTKPREEQYNSTYRVVSVLTVLHQDWLNGKEYKCKVSNKALPAPIEKTISKAKGQPREPQVYTLPPSREEMTKNQVSLTCLVKGFYPSDIAVEWESNGQPENNYKTTPPVLDSDGSFFLYSKLTVDKSRWQQGNVFSCSVMHEALHNHYTQKSLSLSPG

SEQ ID NO: 97 - protein, 119 aa, Artificial Sequence
  Synthetic Construct
EVQLVESGGGLVQPGGSLRLSCAASGYTFTDYNLDWVRQAPGKGLEWVGDINPINGATLYNQKFKGRATISVDQAKNSAYLQMNSLRAEDTAVYYCARYYGDYDAMDYWGQGTLVTVSS

SEQ ID NO: 98 - protein, 448 aa, Artificial Sequence
  Synthetic Construct
EVQLVESGGGLVQPGGSLRLSCAASGYTFTDYNLDWVRQAPGKGLEWVGDINPINGATLYNQKFKGRATISVDQAKNSAYLQMNSLRAEDTAVYYCARYYGDYDAMDYWGQGTLVTVSSASTKGPSVFPLAPSSKSTSGGTAALGCLVKDYFPEPVTVSWNSGALTSGVHTFPAVLQSSGLYSLSSVVTVPSSSLGTQTYICNVNHKPSNTKVDKKVEPKSCDKTHTCPPCPAPEAAGAPSVFLFPPKPKDTLMISRTPEVTCVVVDVSHEDPEVKFNWYVDGVEVHNAKTKPREEQYNSTYRVVSVLTVLHQDWLNGKEYKCKVSNKALPAPIEKTISKAKGQPREPQVYTLPPSREEMTKNQVSLTCLVKGFYPSDIAVEWESNGQPENNYKTTPPVLDSDGSFFLYSKLTVDKSRWQQGNVFSCSVMHEALHNHYTQKSLSLSPG

SEQ ID NO: 99 - protein, 119 aa, Artificial Sequence
  Synthetic Construct
EVQLVESGGGLVQPGGSLRLSCAASGYTFTDYNLDWVRQAPGKGLEWVGDINPINGATLYNQKFKGRFTISRDNAKNSLYLQMNSLRAEDTAVYYCARYYGDYDAMDYWGQGTLVTVSS

SEQ ID NO: 100 - protein, 448 aa, Artificial Sequence
  Synthetic Construct
EVQLVESGGGLVQPGGSLRLSCAASGYTFTDYNLDWVRQAPGKGLEWVGDINPINGATLYNQKFKGRFTISRDNAKNSLYLQMNSLRAEDTAVYYCARYYGDYDAMDYWGQGTLVTVSSASTKGPSVFPLAPSSKSTSGGTAALGCLVKDYFPEPVTVSWNSGALTSGVHTFPAVLQSSGLYSLSSVVTVPSSSLGTQTYICNVNHKPSNTKVDKKVEPKSCDKTHTCPPCPAPEAAGAPSVFLFPPKPKDTLMISRTPEVTCVVVDVSHEDPEVKFNWYVDGVEVHNAKTKPREEQYNSTYRVVSVLTVLHQDWLNGKEYKCKVSNKALPAPIEKTISKAKGQPREPQVYTLPPSREEMTKNQVSLTCLVKGFYPSDIAVEWESNGQPENNYKTTPPVLDSDGSFFLYSKLTVDKSRWQQGNVFSCSVMHEALHNHYTQKSLSLSPG

SEQ ID NO: 101 - protein, 119 aa, Artificial Sequence
  Synthetic Construct
EVQLVESGGGLVQPGGSLRLSCAASGYTFTDYNLDWVRQAPGKGLEWVADINPINGATLYNQKFKGRATISRDNAKNSLYLQMNSLRAEDTAVYYCARYYGDYDAMDYWGQGTLVTVSS

SEQ ID NO: 102 - protein, 448 aa, Artificial Sequence
  Synthetic Construct
EVQLVESGGGLVQPGGSLRLSCAASGYTFTDYNLDWVRQAPGKGLEWVADINPINGATLYNQKFKGRATISRDNAKNSLYLQMNSLRAEDTAVYYCARYYGDYDAMDYWGQGTLVTVSSASTKGPSVFPLAPSSKSTSGGTAALGCLVKDYFPEPVTVSWNSGALTSGVHTFPAVLQSSGLYSLSSVVTVPSSSLGTQTYICNVNHKPSNTKVDKKVEPKSCDKTHTCPPCPAPEAAGAPSVFLFPPKPKDTLMISRTPEVTCVVVDVSHEDPEVKFNWYVDGVEVHNAKTKPREEQYNSTYRVVSVLTVLHQDWLNGKEYKCKVSNKALPAPIEKTISKAKGQPREPQVYTLPPSREEMTKNQVSLTCLVKGFYPSDIAVEWESNGQPENNYKTTPPVLDSDGSFFLYSKLTVDKSRWQQGNVFSCSVMHEALHNHYTQKSLSLSPG

SEQ ID NO: 103 - protein, 119 aa, Artificial Sequence
  Synthetic Construct
EVQLVESGGGLVQPGGSLRLSCAASGYTFTDYNLDWVRQAPGKGLEWVADINPINGATLYNQKFKGRFTISRDQAKNSLYLQMNSLRAEDTAVYYCARYYGDYDAMDYWGQGTLVTVSS

SEQ ID NO: 104 - protein, 448 aa, Artificial Sequence
  Synthetic Construct
EVQLVESGGGLVQPGGSLRLSCAASGYTFTDYNLDWVRQAPGKGLEWVADINPINGATLYNQKFKGRFTISRDQAKNSLYLQMNSLRAEDTAVYYCARYYGDYDAMDYWGQGTLVTVSSASTKGPSVFPLAPSSKSTSGGTAALGCLVKDYFPEPVTVSWNSGALTSGVHTFPAVLQSSGLYSLSSVVTVPSSSLGTQTYICNVNHKPSNTKVDKKVEPKSCDKTHTCPPCPAPEAAGAPSVFLFPPKPKDTLMISRTPEVTCVVVDVSHEDPEVKFNWYVDGVEVHNAKTKPREEQYNSTYRVVSVLTVLHQDWLNGKEYKCKVSNKALPAPIEKTISKAKGQPREPQVYTLPPSREEMTKNQVSLTCLVKGFYPSDIAVEWESNGQPENNYKTTPPVLDSDGSFFLYSKLTVDKSRWQQGNVFSCSVMHEALHNHYTQKSLSLSPG

SEQ ID NO: 105 - protein, 119 aa, Artificial Sequence
  Synthetic Construct
EVQLVESGGGLVQPGGSLRLSCAASGYTFTDYNLDWVRQAPGKGLEWVADINPINGATLYNQKFKGRFTISRDNAKNSAYLQMNSLRAEDTAVYYCARYYGDYDAMDYWGQGTLVTVSS

SEQ ID NO: 106 - protein, 448 aa, Artificial Sequence
  Synthetic Construct
EVQLVESGGGLVQPGGSLRLSCAASGYTFTDYNLDWVRQAPGKGLEWVADINPINGATLYNQKFKGRFTISRDNAKNSAYLQMNSLRAEDTAVYYCARYYGDYDAMDYWGQGTLVTVSSASTKGPSVFPLAPSSKSTSGGTAALGCLVKDYFPEPVTVSWNSGALTSGVHTFPAVLQSSGLYSLSSVVTVPSSSLGTQTYICNVNHKPSNTKVDKKVEPKSCDKTHTCPPCPAPEAAGAPSVFLFPPKPKDTLMISRTPEVTCVVVDVSHEDPEVKFNWYVDGVEVHNAKTKPREEQYNSTYRVVSVLTVLHQDWLNGKEYKCKVSNKALPAPIEKTISKAKGQPREPQVYTLPPSREEMTKNQVSLTCLVKGFYPSDIAVEWESNGQPENNYKTTPPVLDSDGSFFLYSKLTVDKSRWQQGNVFSCSVMHEALHNHYTQKSLSLSPG

SEQ ID NO: 107 - protein, 119 aa, Artificial Sequence
  Synthetic Construct
EVQLVESGGGLVQPGGSLRLSCAASGYTFTDYNLDWVRQAPGKGLEWVGDINPINGATLYNQKFKGRATISVDQAKNSAYLQMNSLRAEDTAVYYCSIYYGDYDAMDYWGQGTLVTVSS

SEQ ID NO: 108 - protein, 448 aa, Artificial Sequence
  Synthetic Construct
EVQLVESGGGLVQPGGSLRLSCAASGYTFTDYNLDWVRQAPGKGLEWVGDINPINGATLYNQKFKGRATISVDQAKNSAYLQMNSLRAEDTAVYYCSIYYGDYDAMDYWGQGTLVTVSSASTKGPSVFPLAPSSKSTSGGTAALGCLVKDYFPEPVTVSWNSGALTSGVHTFPAVLQSSGLYSLSSVVTVPSSSLGTQTYICNVNHKPSNTKVDKKVEPKSCDKTHTCPPCPAPEAAGAPSVFLFPPKPKDTLMISRTPEVTCVVVDVSHEDPEVKFNWYVDGVEVHNAKTKPREEQYNSTYRVVSVLTVLHQDWLNGKEYKCKVSNKALPAPIEKTISKAKGQPREPQVYTLPPSREEMTKNQVSLTCLVKGFYPSDIAVEWESNGQPENNYKTTPPVLDSDGSFFLYSKLTVDKSRWQQGNVFSCSVMHEALHNHYTQKSLSLSPG

SEQ ID NO: 109 - protein, 107 aa, Artificial Sequence
  Synthetic Construct
DIQMTQSPSSLSASVGDRVTITCKASQDVHTAVAWYQQKPGKAPKLLIYWASTRHTGVPSRFSGSGSGTDFTLTISSLQPEDFATYYCQQHYTTPYTFGQGTKLEIK

SEQ ID NO: 110 - protein, 214 aa, Artificial Sequence
  Synthetic Construct
DIQMTQSPSSLSASVGDRVTITCKASQDVHTAVAWYQQKPGKAPKLLIYWASTRHTGVPSRFSGSGSGTDFTLTISSLQPEDFATYYCQQHYTTPYTFGQGTKLEIKRTVAAPSVFIFPPSDEQLKSGTASVVCLLNNFYPREAKVQWKVDNALQSGNSQESVTEQDSKDSTYSLSSTLTLSKADYEKHKVYACEVTHQGLSSPVTKSFNRGEC

SEQ ID NO: 111 - protein, 107 aa, Artificial Sequence
  Synthetic Construct
DIQMTQSPSSLSASVGDRVTITCKASQDVHTAVAWYQQKPGKAPKLLIYWASTRHTGVPSRFSGSGSGTDYTLTISSLQPEDFATYYCQQHYTTPYTFGQGTKLEIK

SEQ ID NO: 112 - protein, 214 aa, Artificial Sequence
  Synthetic Construct
DIQMTQSPSSLSASVGDRVTITCKASQDVHTAVAWYQQKPGKAPKLLIYWASTRHTGVPSRFSGSGSGTDYTLTISSLQPEDFATYYCQQHYTTPYTFGQGTKLEIKRTVAAPSVFIFPPSDEQLKSGTASVVCLLNNFYPREAKVQWKVDNALQSGNSQESVTEQDSKDSTYSLSSTLTLSKADYEKHKVYACEVTHQGLSSPVTKSFNRGEC

SEQ ID NO: 113 - protein, 11 aa, Artificial Sequence
  Synthetic Construct
KASQDVITAVA

SEQ ID NO: 114 - protein, 7 aa, Artificial Sequence
  Synthetic Construct
WASTRHT

SEQ ID NO: 115 - protein, 9 aa, Artificial Sequence
  Synthetic Construct
QQHYSTPYT

SEQ ID NO: 116 - protein, 107 aa, Artificial Sequence
  Synthetic Construct
DIVMTQSHKFMSTSVGDRVSITCKASQDVITAVAWYQQKPGQSPKLLIYWASTRHTGVPVRFTGSGSGTDYTLTIISVQAEDLALYYCQQHYSTPYTFGGGTKLEIK

SEQ ID NO: 117 - protein, 213 aa, Artificial Sequence
  Synthetic Construct
DIVMTQSHKFMSTSVGDRVSITCKASQDVITAVAWYQQKPGQSPKLLIYWASTRHTGVPVRFTGSGSGTDYTLTIISVQAEDLALYYCQQHYSTPYTFGGGTKLEIKADAAPTVSIFPPSSEQLTSGGASVVCFLNNFYPKDINVKWKIDGSERQNGVLNSWTDQDSKDSTYSMSSTLTLTKDEYERHNSYTCEATHKTSTSPIVKSFNRNEC

SEQ ID NO: 118 - protein, 10 aa, Artificial Sequence
  Synthetic Construct
GYTFTDYTMD

SEQ ID NO: 119 - protein, 17 aa, Artificial Sequence
  Synthetic Construct
DINPSNGGSIYNRKFKG

SEQ ID NO: 120 - protein, 10 aa, Artificial Sequence
  Synthetic Construct
MHYNYDGFPY

SEQ ID NO: 121 - protein, 119 aa, Artificial Sequence
  Synthetic Construct
EVLLQQSGPELVKPGSSVKIPCKASGYTFTDYTMDWVKQSHGKSLEWIGDINPSNGGSIYNRKFKGKATLTVDKSSSTAYMELRSLTSEDTAVYYCARMHYNYDGFPYWGQGTLVTVSA

SEQ ID NO: 122 - protein, 448 aa, Artificial Sequence
  Synthetic Construct
EVLLQQSGPELVKPGSSVKIPCKASGYTFTDYTMDWVKQSHGKSLEWIGDINPSNGGSIYNRKFKGKATLTVDKSSSTAYMELRSLTSEDTAVYYCARMHYNYDGFPYWGQGTLVTVSAASTKGPSVFPLAPSSKSTSGGTAALGCLVKDYFPEPVTVSWNSGALTSGVHTFPAVLQSSGLYSLSSVVTVPSSSLGTQTYICNVNHKPSNTKVDKKVEPKSCDKTHTCPPCPAPEAAGAPSVFLFPPKPKDTLMISRTPEVTCVVVDVSHEDPEVKFNWYVDGVEVHNAKTKPREEQYNSTYRVVSVLTVLHQDWLNGKEYKCKVSNKALPAPIEKTISKAKGQPREPQVYTLPPSREEMTKNQVSLTCLVKGFYPSDIAVEWESNGQPENNYKTTPPVLDSDGSFFLYSKLTVDKSRWQQGNVFSCSVMHEALHNHYTQKSLSLSPG

SEQ ID NO: 123 - protein, 15 aa, Artificial Sequence
  Synthetic Construct
RASKSVSTSGYTYMH

SEQ ID NO: 124 - protein, 7 aa, Artificial Sequence
  Synthetic Construct
LASNLES

SEQ ID NO: 125 - protein, 9 aa, Artificial Sequence
  Synthetic Construct
QHIRELPFT

SEQ ID NO: 126 - protein, 111 aa, Artificial Sequence
  Synthetic Construct
DIVLTQSPASLAVSLGQRATISCRASKSVSTSGYTYMHWYQQKPGQPPKLLIYLASNLESGVPARFSGSGSGTDFTLNIHPVEEEDAAAYYCQHIRELPFTFGSGTKLEIK

SEQ ID NO: 127 - protein, 217 aa, Artificial Sequence
  Synthetic Construct
DIVLTQSPASLAVSLGQRATISCRASKSVSTSGYTYMHWYQQKPGQPPKLLIYLASNLESGVPARFSGSGSGTDFTLNIHPVEEEDAAAYYCQHIRELPFTFGSGTKLEIKADAAPTVSIFPPSSEQLTSGGASVVCFLNNFYPKDINVKWKIDGSERQNGVLNSWTDQDSKDSTYSMSSTLTLTKDEYERHNSYTCEATHKTSTSPIVKSFNRNEC

SEQ ID NO: 128 - protein, 10 aa, Artificial Sequence
  Synthetic Construct
GYTFTSYVMH

SEQ ID NO: 129 - protein, 17 aa, Artificial Sequence
  Synthetic Construct
YLNPYNDGTKYNEKFKG

SEQ ID NO: 130 - protein, 8 aa, Artificial Sequence
  Synthetic Construct
TLLYAMDY

SEQ ID NO: 131 - protein, 117 aa, Artificial Sequence
  Synthetic Construct
EVQLQQSGPELVKPGASVKMSCKASGYTFTSYVMHWVKQKPGQGLEWIGYLNPYNDGTKYNEKFKGKASLISDKSSSTVYMELSSLTSEDSAVYYCATTLLYAMDYWGQGSSVTVSS

SEQ ID NO: 132 - protein, 358 aa, Artificial Sequence
  Synthetic Construct
EVQLQQSGPELVKPGASVKMSCKASGYTFTSYVMHWVKQKPGQGLEWIGYLNPYNDGTKYNEKFKGKASLISDKSSSTVYMELSSLTSEDSAVYYCATTLLYAMDYWGQGSSVTVSSASTKGPSVFPLAPSSKSTSGGTAALGCLVKDYFPEPVTVSWNSGALTSGVHTFPAVLQSSGLYSLSSVVTVPSSSLGTQTYICNVNHKPSNTKVDKKVEPKSCDKTHTCPPCPAPEAAGAPSVFLFPPKPKDTLMISRTPEVTCVVVDVSHEDPEVKFNWYVDGVEVHNAKTKPREEQYNSTYRVVSVLTVLHQDWLNGKEYKCKVSNKALPAPIEKTISKAKGQPREPQVYTLPPSREEM

SEQ ID NO: 133 - protein, 11 aa, Artificial Sequence
  Synthetic Construct
SGDNLRNYYAH

SEQ ID NO: 134 - protein, 7 aa, Artificial Sequence
  Synthetic Construct
YDNNRPS

SEQ ID NO: 135 - protein, 9 aa, Artificial Sequence
  Synthetic Construct
QSWDDGVPV

SEQ ID NO: 136 - protein, 107 aa, Artificial Sequence
  Synthetic Construct
DIELTQPPSVSVAPGQTARISCSGDNLRNYYAHWYQQKPGQAPVVVIYYDNNRPSGIPERFSGSNSGNTATLTISGTQAEDEADYYCQSWDDGVPVFGGGTKLTVLG

SEQ ID NO: 137 - protein, 212 aa, Artificial Sequence
  Synthetic Construct
DIELTQPPSVSVAPGQTARISCSGDNLRNYYAHWYQQKPGQAPVVVIYYDNNRPSGIPERFSGSNSGNTATLTISGTQAEDEADYYCQSWDDGVPVFGGGTKLTVLGQPKAAPSVTLFPPSSEELQANKATLVCLISDFYPGAVTVAWKADSSPVKAGVETTTPSKQSNNKYAASSYLSLTPEQWKSHRSYSCQVTHEGSTVEKTVAPTECS

SEQ ID NO: 138 - protein, 10 aa, Artificial Sequence
  Synthetic Construct
GFTFRSYGMS

SEQ ID NO: 139 - protein, 17 aa, Artificial Sequence
  Synthetic Construct
SIRGSSSSTYYADSVKG

SEQ ID NO: 140 - protein, 8 aa, Artificial Sequence
  Synthetic Construct
KYRYWFDY

SEQ ID NO: 141 - protein, 117 aa, Artificial Sequence
  Synthetic Construct
QVQLVESGGGLVQPGGSLRLSCAASGFTFRSYGMSWVRQAPGKGLEWVSSIRGSSSSTYYADSVKGRFTISRDNSKNTLYLQMNSLRAEDTAVYYCARKYRYWFDYWGQGTLVTVSS

SEQ ID NO: 142 - protein, 446 aa, Artificial Sequence
  Synthetic Construct
QVQLVESGGGLVQPGGSLRLSCAASGFTFRSYGMSWVRQAPGKGLEWVSSIRGSSSSTYYADSVKGRFTISRDNSKNTLYLQMNSLRAEDTAVYYCARKYRYWFDYWGQGTLVTVSSASTKGPSVFPLAPSSKSTSGGTAALGCLVKDYFPEPVTVSWNSGALTSGVHTFPAVLQSSGLYSLSSVVTVPSSSLGTQTYICNVNHKPSNTKVDKKVEPKSCDKTHTCPPCPAPEAAGAPSVFLFPPKPKDTLMISRTPEVTCVVVDVSHEDPEVKFNWYVDGVEVHNAKTKPREEQYNSTYRVVSVLTVLHQDWLNGKEYKCKVSNKALPAPIEKTISKAKGQPREPQVYTLPPSREEMTKNQVSLTCLVKGFYPSDIAVEWESNGQPENNYKTTPPVLDSDGSFFLYSKLTVDKSRWQQGNVFSCSVMHEALHNHYTQKSLSLSPG

SEQ ID NO: 143 - protein, 11 aa, Artificial Sequence
  Synthetic Construct
SGDNLRNYYAH

SEQ ID NO: 144 - protein, 7 aa, Artificial Sequence
  Synthetic Construct
YDVNRPS

SEQ ID NO: 145 - protein, 9 aa, Artificial Sequence
  Synthetic Construct
QSWWDGVPV

SEQ ID NO: 146 - protein, 107 aa, Artificial Sequence
  Synthetic Construct
DIELTQPPSVSVAPGQTARISCSGDNLRNYYAHWYQQKPGQAPVVVIFYDVNRPSGIPERFSGSNSGNTATLTISGTQAEDEADYYCQSWWDGVPVFGGGTKLTVLG

SEQ ID NO: 147 - protein, 212 aa, Artificial Sequence
  Synthetic Construct
DIELTQPPSVSVAPGQTARISCSGDNLRNYYAHWYQQKPGQAPVVVIFYDVNRPSGIPERFSGSNSGNTATLTISGTQAEDEADYYCQSWWDGVPVFGGGTKLTVLGQPKAAPSVTLFPPSSEELQANKATLVCLISDFYPGAVTVAWKADSSPVKAGVETTTPSKQSNNKYAASSYLSLTPEQWKSHRSYSCQVTHEGSTVEKTVAPTECS

SEQ ID NO: 148 - protein, 10 aa, Artificial Sequence
  Synthetic Construct
GFTFRSYGMD

SEQ ID NO: 149 - protein, 17 aa, Artificial Sequence
  Synthetic Construct
SIRGSRSSTYYADSVKG

SEQ ID NO: 150 - protein, 8 aa, Artificial Sequence
  Synthetic Construct
LYRYWFDY

SEQ ID NO: 151 - protein, 117 aa, Artificial Sequence
  Synthetic Construct
QVQLVESGGGLVQPGGSLRLSCAASGFTFRSYGMDWVRQAPGKGLEWVSSIRGSRSSTYYADSVKGRFTISRDNSKNTLYLQMNSLRAEDTAVYYCARLYRYWFDYWGQGTLVTVSS

SEQ ID NO: 152 - protein, 446 aa, Artificial Sequence
  Synthetic Construct
QVQLVESGGGLVQPGGSLRLSCAASGFTFRSYGMDWVRQAPGKGLEWVSSIRGSRSSTYYADSVKGRFTISRDNSKNTLYLQMNSLRAEDTAVYYCARLYRYWFDYWGQGTLVTVSSASTKGPSVFPLAPSSKSTSGGTAALGCLVKDYFPEPVTVSWNSGALTSGVHTFPAVLQSSGLYSLSSVVTVPSSSLGTQTYICNVNHKPSNTKVDKKVEPKSCDKTHTCPPCPAPEAAGAPSVFLFPPKPKDTLMISRTPEVTCVVVDVSHEDPEVKFNWYVDGVEVHNAKTKPREEQYNSTYRVVSVLTVLHQDWLNGKEYKCKVSNKALPAPIEKTISKAKGQPREPQVYTLPPSREEMTKNQVSLTCLVKGFYPSDIAVEWESNGQPENNYKTTPPVLDSDGSFFLYSKLTVDKSRWQQGNVFSCSVMHEALHNHYTQKSLSLSPG

SEQ ID NO: 153 - protein, 11 aa, Artificial Sequence
  Synthetic Construct
SGDNLRNYYAH

SEQ ID NO: 154 - protein, 7 aa, Artificial Sequence
  Synthetic Construct
YDNNRPS

SEQ ID NO: 155 - protein, 9 aa, Artificial Sequence
  Synthetic Construct
QSWDDGVPV

SEQ ID NO: 156 - protein, 107 aa, Artificial Sequence; identical to SEQ ID NO: 136
  Synthetic Construct

SEQ ID NO: 157 - protein, 105 aa, Artificial Sequence; identical to SEQ ID NO: 26
  Synthetic Construct

SEQ ID NO: 158 - protein, 212 aa, Artificial Sequence; identical to SEQ ID NO: 137
  Synthetic Construct

SEQ ID NO: 159 - protein, 10 aa, Artificial Sequence
  Synthetic Construct
GFTFSNYALS

SEQ ID NO: 160 - protein, 16 aa, Artificial Sequence
  Synthetic Construct
SISSGGATYYPDSVEG

SEQ ID NO: 161 - protein, 10 aa, Artificial Sequence
  Synthetic Construct
GAYGSDYFDY

SEQ ID NO: 162 - protein, 118 aa, Artificial Sequence
  Synthetic Construct
EVKLVESGGGLVKPGGSLRLSCAASGFTFSNYALSWVRQTPDKRLEWVASISSGGATYYPDSVEGRFTISRDNVRNILYLQMSSLQSEDTAMYYCTRGAYGSDYFDYWGQGTTLTVSS

SEQ ID NO: 163 - protein, 441 aa, Artificial Sequence
  Synthetic Construct
EVKLVESGGGLVKPGGSLRLSCAASGFTFSNYALSWVRQTPDKRLEWVASISSGGATYYPDSVEGRFTISRDNVRNILYLQMSSLQSEDTAMYYCTRGAYGSDYFDYWGQGTTLTVSSAKTTPPSVYPLAPGSAAQTNSMVTLGCLVKGYFPEPVTVTWNSGSLSSGVHTFPAVLQSDLYTLSSSVTVPSSTWPSETVTCNVAHPASSTKVDKKIVPRDCGCKPCICTVPEVSSVFIFPPKPKDVLTITLTPKVTCVVVDISKDDPEVQFSWFVDDVEVHTAQTQPREEQFNSTFRSVSELPIMHQDWLNGKEFKCRVNSAAFPAPIEKTISKTKGRPKAPQVYTIPPPKEQMAKDKVSLTCMITDFFPEDITVEWQWNGQPAENYKNTQPIMDTDGSYFVYSKLNVQKSNWEAGNTFTCSVLHEGLHNHHTEKSLSHSPG

SEQ ID NO: 164 - protein, 16 aa, Artificial Sequence
  Synthetic Construct
KSSQSLLESDGKTYLN

SEQ ID NO: 165 - protein, 7 aa, Artificial Sequence
  Synthetic Construct
LVSILDS

SEQ ID NO: 166 - protein, 9 aa, Artificial Sequence
  Synthetic Construct
LQATHFPQT

SEQ ID NO: 167 - protein, 112 aa, Artificial Sequence [sequence omitted]

SEQ ID NO: 168 - protein, 219 aa, Artificial Sequence
  Synthetic Construct
DIVMTQTPLSLSVTPGQPASISCKSSQSLLESDGKTYLNWYLQKPGQSPQLLIYLVSILDSGVPDRFSGSGSGTDFTLKISRVEAEDVGVYYCLQATHFPQTFGGGTKVEIKRTVAAPSVFIFPPSDEQLKSGTASVVCLLNNFYPREAKVQWKVDNALQSGNSQESVTEQDSKDSTYSLSSTLTLSKADYEKHKVYACEVTHQGLSSPVTKSFNRGEC

SEQ ID NO: 169 - protein, 10 aa, Artificial Sequence
  Synthetic Construct
GFTFSNYAMS

SEQ ID NO: 170 - protein, 17 aa, Artificial Sequence
  Synthetic Construct
TISRSGSYSYFPDSVQG

SEQ ID NO: 171 - protein, 12 aa, Artificial Sequence
  Synthetic Construct
LGGYDEGDAMDS

SEQ ID NO: 172 - protein, 121 aa, Artificial Sequence [sequence omitted]

SEQ ID NO: 173 - protein, 327 aa, Artificial Sequence
  Synthetic Construct
ASTKGPSVFPLAPCSRSTSESTAALGCLVKDYFPEPVTVSWNSGALTSGVHTFPAVLQSSGLYSLSSVVTVPSSSLGTKTYTCNVDHKPSNTKVDKRVESKYGPPCPPCPAPEFLGGPSVFLFPPKPKDTLMISRTPEVTCVVVDVSQEDPEVQFNWYVDGVEVHNAKTKPREEQFNSTYRVVSVLTVLHQDWLNGKEYKCKVSNKGLPSSIEKTISKAKGQPREPQVYTLPPSQEEMTKNQVSLTCLVKGFYPSDIAVEWESNGQPENNYKTTPPVLDSDGSFFLYSRLTVDKSRWQEGNVFSCSVMHEALHNHYTQKSLSLSLGK

SEQ ID NO: 174 - protein, 448 aa, Artificial Sequence
  Synthetic Construct
EVQLVESGGGLVKPGGSLRLSCAASGFTFSNYAMSWVRQTPEKRLEWVATISRSGSYSYFPDSVQGRFTISRDNAKNSLYLQMNSLRAEDTAVYYCARLGGYDEGDAMDSWGQGTTVTVSSASTKGPSVFPLAPCSRSTSESTAALGCLVKDYFPEPVTVSWNSGALTSGVHTFPAVLQSSGLYSLSSVVTVPSSSLGTKTYTCNVDHKPSNTKVDKRVESKYGPPCPPCPAPEFLGGPSVFLFPPKPKDTLMISRTPEVTCVVVDVSQEDPEVQFNWYVDGVEVHNAKTKPREEQFNSTYRVVSVLTVLHQDWLNGKEYKCKVSNKGLPSSIEKTISKAKGQPREPQVYTLPPSQEEMTKNQVSLTCLVKGFYPSDIAVEWESNGQPENNYKTTPPVLDSDGSFFLYSRLTVDKSRWQEGNVFSCSVMHEALHNHYTQKSLSLSLGK

SEQ ID NO: 175 - DNA, 360 bp, Artificial Sequence
  Synthetic Construct
gaggtgcagctgctggagtctggcggaggcttggtacagcctggggggtccctgagactctcctgtgcagcctctggattcacctttagcagctatgccatgagctgggtccgccaggctccagggaaggggctggagtgggtctcagctattagtggtagtggtggtagcacatactacgcagactccgtgaagggccggttcaccatctccagagacaattccaagaacacgctgtatctgcaaatgaacagcctgagagccgaggacacggccgtatattactgtgcgattctgggagctacttcgttatcggcttttgatatctggggccaagggacaatggtcaccgtctcgagc

SEQ ID NO: 176 - DNA, 336 bp, Artificial Sequence
  Synthetic Construct
cagtctgtgctgacgcagccgccctcagtgtctggggccccagggcagagggtcaccatctcctgcactgggagcagctccaacatcggggcaggttatgatgtacactggtaccagcagcttccaggaacagcccccaaactcctcatctatggtaacagcaatcggccctcaggggtccctgaccgattctctggctccaagtctggcacctcagcctccctggccatcactgggctccaggctgaggatgaggctgattattactgccagtcctatgacagcagcctgagtggttcaggggtattcggcggagggaccaagctgaccgtccta

SEQ ID NO: 177 - DNA, 1347 bp, Artificial Sequence
  Synthetic Construct
gaggtgcagctgctggagtctggcggaggcttggtacagcctggggggtccctgagactctcctgtgcagcctctggattcacctttagcagctatgccatgagctgggtccgccaggctccagggaaggggctggagtgggtctcagctattagtggtagtggtggtagcacatactacgcagactccgtgaagggccggttcaccatctccagagacaattccaagaacacgctgtatctgcaaatgaacagcctgagagccgaggacacggccgtatattactgtgcgattctgggagctacttcgttatcggcttttgatatctggggccaagggacaatggtcaccgtctcgagcgcgtcgaccaagggcccatcggtcttccccctggcaccctcctccaagagcacctctgggggcacagcggccctgggctgcctggtcaaggactacttccccgaaccggtgacggtgtcgtggaactcaggcgccctgaccagcggcgtgcacaccttcccggctgtcctacagtcctcaggactctactccctcagcagcgtggtgaccgtgccctccagcagcttgggcacccagacctacatctgcaacgtgaatcacaagcccagcaacaccaaggtggacaagaaagttgagcccaaatcttgtgacaaaactcacacatgcccaccgtgcccagcacctgaagccgctggggcaccgtcagtcttcctcttccccccaaaacccaaggacaccctcatgatctcccggacccctgaggtcacatgcgtggtggtggacgtgagccacgaagaccctgaggtcaagttcaactggtacgtggacggcgtggaggtgcataatgccaagacaaagccgcgggaggagcagtacaacagcacgtaccgtgtggtcagcgtcctcaccgtcctgcaccaggactggctgaatggcaaggagtacaagtgcaaggtctccaacaaagccctcccagcccccatcgagaaaaccatctccaaagccaaagggcagccccgagaaccacaggtgtacaccctgcccccatcccgggaggagatgaccaagaaccaggtcagcctgacctgcctggtcaaaggcttctatcccagcgacatcgccgtggagtgggagagcaatgggcagccggagaacaactacaagaccacgcctcccgtgctggactccgacggctccttcttcctctatagcaagctcaccgtggacaagagcaggtggcagcaggggaacgtcttctcatgctccgtgatgcatgaggctctgcacaaccactacacgcagaagagcctctccctgtccccgggt

SEQ ID NO: 178 - DNA, 654 bp, Artificial Sequence
  Synthetic Construct
cagtctgtgctgacgcagccgccctcagtgtctggggccccagggcagagggtcaccatctcctgcactgggagcagctccaacatcggggcaggttatgatgtacactggtaccagcagcttccaggaacagcccccaaactcctcatctatggtaacagcaatcggccctcaggggtccctgaccgattctctggctccaagtctggcacctcagcctccctggccatcactgggctccaggctgaggatgaggctgattattactgccagtcctatgacagcagcctgagtggttcaggggtattcggcggagggaccaagctgaccgtcctaggtcagcccaaggctgccccctcggtcactctgttcccgccctcctctgaggagcttcaagccaacaaggccacactggtgtgtctcataagtgacttctacccgggagccgtgacagtggcctggaaggcagatagcagccccgtcaaggcgggagtggagaccaccacaccctccaaacaaagcaacaacaagtacgcggccagcagctatctgagcctgacgcctgagcagtggaagtcccacagaagctacagctgccaggtcacgcatgaagggagcaccgtggagaagacagtggcccctacagaatgttca